European Patent Application EP 4 644 550 A1, published November 5, 2025. Title: VACCINE AGAINST RESPIRATORY SYNCYTIAL VIRUS INFECTION. Applicant: WestVac Biopharma Co., Ltd. Application CN. The sequence listing filed with the application follows.

SEQUENCE LISTING (39 sequences)

SEQ ID NO: 1 - protein, 549 aa, synthetic construct
QNITEEFYQSTCSAVSKGYLSALRTGWYTSVITIELSNIKENKCNGTDAKVKLIKQELDKYKNAVTELQLLMQSTPPTNNRARRELPRFMNYTLNNAKKTNVTLSKKRKRRFLGFLLGVGSAIASGVAVSKVLHLEGEVNKIKSALLSTNKAVVSLSNGVSVLTSKVLDLKNYIDKQLLPIVNKQSCSISNIETVIEFQQKNNRLLEITREFSVNAGVTTPVSTYMLTNSELLSLINDMPITNDQKKLMSNNVQIVRQQSYSIMSIIKEEVLAYVVQLPLYGVIDTPCWKLHTSPLCTTNTKEGSNICLTRTDRGWYCDNAGSVSFFPQAETCKVQSNRVFCDTMNSLTLPSEINLCNVDIFNPKYDCKIMTSKTDVSSSVITSLGAIVSCYGKTKCTASNKNRGIIKTFSNGCDYVSNKGMDTVSVGNTLYYVNKQEGKSLYVKGEPIINFYDPLVFPSDEFDASISQVNEKINQSLAFIRKSDELLHNVNAGKSTTNIMITTIIIVIIVILLSLIAVGLLLYCKARSTPVTLSKDQLSGINNIAFSN

SEQ ID NO: 2 - protein, 549 aa, synthetic construct
QNITEEFYQSTCSAVSRGYFSALRTGWYTSVITIELSNIKETKCNGTDTKVKLIKQELDKYKNAVTELQLLMQNTPAANNRARREAPQYMNYTINTTKNLNVSISKKRKRRFLGFLLGVGSAIASGIAVSKVLHLEGEVNKIKNALLSTNKAVVSLSNGVSVLTSKVLDLKNYINNRLLPIVNQQSCRISNIETVIEFQQMNSRLLEITREFSVNAGVTTPLSTYMLTNSELLSLINDMPITNDQKKLMSSNVQIVRQQSYSIMSIIKEEVLAYVVQLPIYGVIDTPCWKLHTSPLCTTNIKEGSNICLTRTDRGWYCDNAGSVSFFPQADTCKVQSNRVFCDTMNSLTLPSEVSLCNTDIFNSKYDCKIMTSKTDISSSVITSLGAIVSCYGKTKCTASNKNRGIIKTFSNGCDYVSNKGVDTVSVGNTLYYVNKLEGKNLYVKGEPIINYYDPLVFPSDEFDASISQVNEKINQSLAFIRRSDELLHNVNTGKSTTNIMITTIIIVIIVVLLSLIAIGLLLYCKAKNTPVTLSKDQLSGINNIAFSK

SEQ ID NO: 3 - protein, 446 aa, synthetic construct
QNCTEEFYQSTCSAVSKGYLSALRTGWYTCVITIELSNIKENKCNGTDAKVKLIKQELDKYKNAVTELQLLMQSTPPTSAIASGVAVSKVLHLEGEVNKIKSALLSTNKAVVSLSNGVSVCTSKVLDLKNYIDKQLLPIVNKQSCSISNIETVIEFQQKNNRLLEITREFSVNAGVTTPVSTYMLTNSELLSLINDMPITNDQKKLMSNNVQIVRQQSYSIMSIIKEEVLAYVVQLPLYGVIDTPCWKLHTSPLCTTNTKEGSNICLTRTDRGWYCDNAGSVSFFPQAETCKVQSNRVFCDTMNSLTLPSEINLCNVDIFNPKYDCKIMTSKTDVSSSVITSLGAIVSCYGKTKCTASNKNRGIIKTFSNGCDYVSNKGMDTVSVGNTLYYVNKQECKSLYVKGEPIINFYDPLVFPSDEFDASISQVNEKINQSLAFIRKSDELL

SEQ ID NO: 4 - protein, 446 aa, synthetic construct
QNCTEEFYQSTCSAVSRGYFSALRTGWYTCVITIELSNIKETKCNGTDTKVKLIKQELDKYKNAVTELQLLMQNTPAASAIASGIAVSKVLHLEGEVNKIKNALLSTNKAVVSLSNGVSVCTSKVLDLKNYINNRLLPIVNQQSCRISNIETVIEFQQMNSRLLEITREFSVNAGVTTPLSTYMLTNSELLSLINDMPITNDQKKLMSSNVQIVRQQSYSIMSIIKEEVLAYVVQLPIYGVIDTPCWKLHTSPLCTTNIKEGSNICLTRTDRGWYCDNAGSVSFFPQADTCKVQSNRVFCDTMNSLTLPSEVSLCNTDIFNSKYDCKIMTSKTDISSSVITSLGAIVSCYGKTKCTASNKNRGIIKTFSNGCDYVSNKGVDTVSVGNTLYYVNKLECKNLYVKGEPIINYYDPLVFPSDEFDASISQVNEKINQSLAFIRRSDELL

SEQ ID NO: 5 - protein, 477 aa, synthetic construct
QNCTEEFYQSTCSAVSKGYLSALRTGWYTCVITIELSNIKENKCNGTDAKVKLIKQELDKYKNAVTELQLLMQSTPPTSAIASGVAVSKVLHLEGEVNKIKSALLSTNKAVVSLSNGVSVCTSKVLDLKNYIDKQLLPIVNKQSCSISNIETVIEFQQKNNRLLEITREFSVNAGVTTPVSTYMLTNSELLSLINDMPITNDQKKLMSNNVQIVRQQSYSIMSIIKEEVLAYVVQLPLYGVIDTPCWKLHTSPLCTTNTKEGSNICLTRTDRGWYCDNAGSVSFFPQAETCKVQSNRVFCDTMNSLTLPSEINLCNVDIFNPKYDCKIMTSKTDVSSSVITSLGAIVSCYGKTKCTASNKNRGIIKTFSNGCDYVSNKGMDTVSVGNTLYYVNKQECKSLYVKGEPIINFYDPLVFPSDEFDASISQVNEKINQSLAFIRKSDELLSAIGGYIPEAPRDGQAYVRKDGEWVLLSTFL

SEQ ID NO: 6 - protein, 477 aa, synthetic construct
QNCTEEFYQSTCSAVSRGYFSALRTGWYTCVITIELSNIKETKCNGTDTKVKLIKQELDKYKNAVTELQLLMQNTPAASAIASGIAVSKVLHLEGEVNKIKNALLSTNKAVVSLSNGVSVCTSKVLDLKNYINNRLLPIVNQQSCRISNIETVIEFQQMNSRLLEITREFSVNAGVTTPLSTYMLTNSELLSLINDMPITNDQKKLMSSNVQIVRQQSYSIMSIIKEEVLAYVVQLPIYGVIDTPCWKLHTSPLCTTNIKEGSNICLTRTDRGWYCDNAGSVSFFPQADTCKVQSNRVFCDTMNSLTLPSEVSLCNTDIFNSKYDCKIMTSKTDISSSVITSLGAIVSCYGKTKCTASNKNRGIIKTFSNGCDYVSNKGVDTVSVGNTLYYVNKLECKNLYVKGEPIINYYDPLVFPSDEFDASISQVNEKINQSLAFIRRSDELLSAIGGYIPEAPRDGQAYVRKDGEWVLLSTFL

SEQ ID NO: 7 - protein, 523 aa, synthetic construct
MELLILKANAITTILTAVTFCFASGQNCTEEFYQSTCSAVSKGYLSALRTGWYTCVITIELSNIKENKCNGTDAKVKLIKQELDKYKNAVTELQLLMQSTPPTSAIASGVAVSKVLHLEGEVNKIKSALLSTNKAVVSLSNGVSVCTSKVLDLKNYIDKQLLPIVNKQSCSISNIETVIEFQQKNNRLLEITREFSVNAGVTTPVSTYMLTNSELLSLINDMPITNDQKKLMSNNVQIVRQQSYSIMSIIKEEVLAYVVQLPLYGVIDTPCWKLHTSPLCTTNTKEGSNICLTRTDRGWYCDNAGSVSFFPQAETCKVQSNRVFCDTMNSLTLPSEINLCNVDIFNPKYDCKIMTSKTDVSSSVITSLGAIVSCYGKTKCTASNKNRGIIKTFSNGCDYVSNKGMDTVSVGNTLYYVNKQECKSLYVKGEPIINFYDPLVFPSDEFDASISQVNEKINQSLAFIRKSDELLSAIGGYIPEAPRDGQAYVRKDGEWVLLSTFLVPRGSHHHHHHGSWSHPQFEK

SEQ ID NO: 8 - protein, 523 aa, synthetic construct
MELLILKANAITTILTAVTFCFASGQNCTEEFYQSTCSAVSRGYFSALRTGWYTCVITIELSNIKETKCNGTDTKVKLIKQELDKYKNAVTELQLLMQNTPAASAIASGIAVSKVLHLEGEVNKIKNALLSTNKAVVSLSNGVSVCTSKVLDLKNYINNRLLPIVNQQSCRISNIETVIEFQQMNSRLLEITREFSVNAGVTTPLSTYMLTNSELLSLINDMPITNDQKKLMSSNVQIVRQQSYSIMSIIKEEVLAYVVQLPIYGVIDTPCWKLHTSPLCTTNIKEGSNICLTRTDRGWYCDNAGSVSFFPQADTCKVQSNRVFCDTMNSLTLPSEVSLCNTDIFNSKYDCKIMTSKTDISSSVITSLGAIVSCYGKTKCTASNKNRGIIKTFSNGCDYVSNKGVDTVSVGNTLYYVNKLECKNLYVKGEPIINYYDPLVFPSDEFDASISQVNEKINQSLAFIRRSDELLSAIGGYIPEAPRDGQAYVRKDGEWVLLSTFLVPRGSHHHHHHGSWSHPQFEK

SEQ ID NO: 9 - DNA, 1572 bp, synthetic construct
  source 1..1572: mol_type = other DNA
atggagctgctgatcctgaaggccaacgccatcacaaccatcctgacagccgtgacattctgcttcgcctccggccagaattgcaccgaggagttctaccagtccacatgttccgccgtgagcaagggctacctgtccgccctgagaaccggctggtacacctgtgtgatcaccatcgagctgtccaatatcaaggagaacaagtgcaacggcaccgacgccaaggtgaagctgatcaagcaggagctggacaagtacaagaacgccgtgaccgagctgcagctgctgatgcagagcacacctcccacctccgccatcgccagcggcgttgctgtgtccaaggtgctgcacctggagggcgaggtgaacaagatcaagtccgccctgctgtccaccaacaaggccgtggtgtccctgagcaacggcgtgtccgtgtgcaccagcaaggtgctggatctgaagaattacatcgacaagcagctgctgcccatcgtgaataagcagagctgtagcatcagcaacatcgagaccgtgatcgagttccagcagaagaataacaggctgctggagatcaccagggagttctccgtgaacgccggcgtgaccacacccgtgagcacctacatgctgaccaattccgagctgctgtccctgatcaatgatatgcccatcaccaatgatcagaagaagctgatgtccaacaacgtgcagatcgtgaggcagcagtcctacagcatcatgtccatcatcaaggaggaggtgctggcctacgtggtgcagctgcctctgtacggcgtgatcgataccccttgctggaagctgcacaccagccccctgtgcacaacaaacaccaaggagggcagcaacatctgcctgacaaggacagacagaggctggtactgtgataacgccggcagcgtgtccttcttcccccaggccgagacctgcaaggtgcagtccaacagagtgttctgcgataccatgaactccctgaccctgcctagcgagatcaacctgtgcaacgtggatatcttcaatcctaagtacgattgtaagatcatgacctccaagacagacgtgtccagcagcgtgatcacatccctgggcgccatcgtgtcctgttacggcaagaccaagtgtaccgcctccaataagaataggggcatcatcaagacattctccaatggctgcgattacgtgtccaacaagggcatggataccgtgagcgtgggcaatacactgtactacgtgaacaagcaggagtgtaagtccctgtacgtgaagggcgagcctatcatcaacttctacgaccccctggtgttccctagcgacgagttcgacgccagcatctcccaggtgaacgagaagatcaaccagtccctggccttcatcaggaagagcgacgagctgctgagcgccatcggcggctacatccctgaggcccctagggacggccaggcctacgtgaggaaggacggcgagtgggtgctgctgtccacattcctggtgcctagaggctcccaccaccaccaccatcacggcagctggtcccaccctcagttcgagaagtga

SEQ ID NO: 10 - DNA, 1572 bp, synthetic construct
  source 1..1572: mol_type = other DNA
atggagctgctgatccacaggagcagcgccatcttcctgaccctggccgtgaacgccctgtacctgacaagctcccagaactgcaccgaggagttctaccagagcacctgtagcgccgtgtccaggggctacttcagcgccctgaggaccggctggtacacctgcgtgatcaccatcgagctgtccaatatcaaggagaccaagtgtaacggcaccgataccaaggtgaagctgatcaagcaggagctggataagtacaagaatgccgtgaccgagctgcagctgctgatgcagaatacacctgccgcctccgccatcgccagcggaatcgctgtgtccaaggtgctgcacctggagggcgaggtgaataagatcaagaatgccctgctgtccacaaacaaggccgtggtgagcctgagcaacggcgtgagcgtgtgtacatccaaggtgctcgacctgaagaactacatcaacaatagactgctgcctatcgtgaaccagcagagctgtaggatcagcaatatcgagacagtgatcgagttccagcagatgaacagcaggctgctggagatcacaagagagttctccgtgaatgccggcgtgacaacacctctgtccacctacatgctgacaaattccgagctgctgtccctgatcaatgatatgcctatcacaaacgatcagaagaagctgatgagctccaatgtgcagatcgtgaggcagcagagctactccatcatgtccatcatcaaggaggaggtgctggcctacgtggtgcagctgcccatctacggcgtgatcgacaccccctgctggaagctgcacacatcccctctgtgcaccaccaatatcaaggaaggctccaatatctgtctgaccaggaccgataggggctggtactgcgataatgccggctccgtgagcttcttccctcaggccgacacctgtaaggtgcagagcaatagagtgttctgtgataccatgaactccctgaccctgccctccgaggtgagcctgtgtaatacagatatcttcaatagcaagtacgattgcaagatcatgaccagcaagaccgatatctccagcagcgtgatcacctccctgggcgccatcgtgagctgctacggcaagaccaagtgtaccgcctccaacaagaacagaggcatcatcaagaccttcagcaatggctgtgactacgtgagcaacaagggcgtggacaccgtgagcgtgggcaatacactgtactacgtgaacaagctggagtgtaagaacctgtacgtgaagggcgagcctatcatcaattactacgaccctctggtgttcccctccgatgagttcgacgccagcatctcccaggtgaacgagaagatcaatcagtccctggccttcatcagaagatccgatgagctgctgagcgccatcggcggctacatccccgaggcccctagagatggccaggcctacgtgagaaaggatggcgagtgggtgctgctgtccaccttcctggtgcccaggggcagccaccaccaccaccatcacggctcctggtcccacccccagttcgagaagtga

SEQ ID NO: 11 - protein, 502 aa, synthetic construct
MELLILKANAITTILTAVTFCFASGQNITEEFYQSTCSAVSKGYLSALRTGWYTSVITIELSNIKENKCNGTDAKVKLIKQELDKYKNAVTELQLLMQSTPPTSAIASGVAVSKVLHLEGEVNKIKSALLSTNKAVVSLSNGVSVLTSKVLDLKNYIDKQLLPIVNKQSCSISNIETVIEFQQKNNRLLEITREFSVNAGVTTPVSTYMLTNSELLSLINDMPITNDQKKLMSNNVQIVRQQSYSIMSIIKEEVLAYVVQLPLYGVIDTPCWKLHTSPLCTTNTKEGSNICLTRTDRGWYCDNAGSVSFFPQAETCKVQSNRVFCDTMNSLTLPSEINLCNVDIFNPKYDCKIMTSKTDVSSSVITSLGAIVSCYGKTKCTASNKNRGIIKTFSNGCDYVSNKGMDTVSVGNTLYYVNKQEGKSLYVKGEPIINFYDPLVFPSDEFDASISQVNEKINQSLAFIRKSDELLSAIGGYIPEAPRDGQAYVRKDGEWVLLSTFL

SEQ ID NO: 12 - DNA, 1509 bp, synthetic construct
  source 1..1509: mol_type = other DNA
atggagctgctgatcctgaaggccaacgccatcaccaccatcctgaccgccgtgaccttctgcttcgctagcgggcagaacatcaccgaggagttctatcagagcacctgcagcgctgtgagcaaaggctatctgagcgccctgagaaccggctggtacacaagcgtcatcaccatcgagctgagcaacatcaaggagaacaagtgcaacggcaccgacgccaaggtgaagctgatcaagcaagagctggacaagtacaagaacgccgtgaccgagctgcagctcctgatgcagagcaccccccctacctccgctattgctagcggcgtggccgtgagcaaggtcctgcacctggagggcgaggtgaacaagatcaagagcgccctgctcagcaccaacaaggccgtggtgagcctgagcaacggcgtgagcgtgctgacaagcaaggtgctggacctgaagaactacatcgacaagcagctgctgcccatcgtgaacaagcagagctgcagcatcagcaacatcgagaccgtgatcgagtttcagcagaagaacaacagactgctggagatcacaagagagttcagcgtgaacgccggcgtgaccacccccgtgagcacctacatgctgaccaacagcgaactgctgtccctgattaacgacatgcccatcaccaacgatcagaagaagctgatgagcaacaacgtgcagatcgtgagacagcagagctacagcatcatgagcatcatcaaggaagaggtgctggcctacgtggtgcagctgcccctgtacggcgtgatcgacaccccctgctggaagctgcacacaagccccctgtgcaccaccaacaccaaggagggcagcaacatctgcctgacaagaaccgacagaggctggtactgcgacaacgccggcagcgtgagcttcttcccccaagccgagacctgcaaggtgcagagcaacagagtgttctgcgacaccatgaacagcctgaccctgcctagcgagatcaacctgtgcaacgtggacatcttcaaccccaagtacgactgcaagatcatgacaagcaagaccgacgtgagcagcagcgtgatcacaagcctgggcgccatcgtgagctgctacggcaagaccaagtgcaccgctagcaacaagaacagaggcatcatcaagaccttcagcaacggctgcgactacgtgagcaacaagggcatggacaccgtgagcgtgggcaacaccctgtactacgtcaacaagcaagaggggaagagcctgtacgtgaagggcgagcccatcatcaacttctacgaccccctggtgttccctagcgacgagttcgacgctagcatcagccaagtgaacgagaagatcaatcagagcctggccttcatcagaaagagcgacgagctgctgagcgctatcggcggctacatccccgaggcccctagagacggccaagcctacgtgagaaaggacggcgagtgggtgctgctgtccaccttcctctga

SEQ ID NO: 13 - protein, 532 aa, synthetic construct
MELLILKANAITTILTAVTFCFASGQNITEEFYQSTCSAVSKGYLSALRTGWYTSVITIELSNIKENKCNGTDAKVKLIKQELDKYKNAVTELQLLMQSTPPTSAIASGVAVSKVLHLEGEVNKIKSALLSTNKAVVSLSNGVSVLTSKVLDLKNYIDKQLLPIVNKQSCSISNIETVIEFQQKNNRLLEITREFSVNAGVTTPVSTYMLTNSELLSLINDMPITNDQKKLMSNNVQIVRQQSYSIMSIIKEEVLAYVVQLPLYGVIDTPCWKLHTSPLCTTNTKEGSNICLTRTDRGWYCDNAGSVSFFPQAETCKVQSNRVFCDTMNSLTLPSEINLCNVDIFNPKYDCKIMTSKTDVSSSVITSLGAIVSCYGKTKCTASNKNRGIIKTFSNGCDYVSNKGMDTVSVGNTLYYVNKQEGKSLYVKGEPIINFYDPLVFPSDEFDASISQVNEKINQSLAFIRKSDELLHNVNAGKSTTNIMITTIIIVIIVILLSLIAVGLLLYCKARSTPVTLSKDQLSGINNIAFSN

SEQ ID NO: 14 - DNA, 1599 bp, synthetic construct
  source 1..1599: mol_type = other DNA
atggagctgctgatcctgaaggccaacgccatcacaaccatcctgaccgccgtgaccttctgcttcgctagcgggcagaacatcaccgaggagttctatcagagcacctgcagcgccgtgagcaaggggtatctgagcgccctgagaaccggctggtacacctccgtcatcaccatcgagctgagcaacatcaaggagaacaagtgcaacggcaccgacgccaaggtgaagctgatcaagcaagagctggacaagtacaagaacgccgtgaccgagctgcaactgctgatgcaaagcacccctcccacaagcgccatcgcctccggcgtggctgtcagcaaggtcctccatctggagggcgaggtgaacaagatcaagagcgccctgctgagcaccaacaaggccgtggtgagcctgagcaacggcgtgagcgtgctgacctccaaggtgctggatctgaagaactacatcgacaagcagctgctgcccatcgtgaacaagcagagctgcagcatcagcaacatcgagaccgtgatcgagtttcagcagaagaacaacagactgctggagatcacaagagagttcagcgtgaatgctggcgtcaccacccccgtgagcacctacatgctgaccaacagcgagctgctgagcctgatcaacgacatgcccatcaccaacgatcagaagaagctgatgagcaacaacgtgcagatcgtgagacagcagagctacagcatcatgagcatcatcaaggaagaggtgctggcctacgtggtgcagctgcccctgtacggcgtgatcgacaccccctgctggaagctgcacacaagccccctgtgcacaaccaacaccaaggagggcagcaacatctgcctgacaagaaccgacagaggctggtactgcgacaacgccggcagcgtgagcttcttcccccaagccgagacctgcaaggtgcagagcaacagagtgttctgcgacaccatgaacagcctgaccctgcctagcgagatcaacctgtgcaacgtggacatcttcaaccccaagtacgactgcaagatcatgacaagcaagaccgacgtgagcagcagcgtgattacaagcctgggcgccatcgtgagctgctacggcaagaccaagtgcaccgctagcaacaagaacagaggcatcatcaagaccttcagcaacggctgcgactacgtgagcaacaagggcatggacaccgtgagcgtgggcaacaccctgtactacgtgaataagcaagagggcaagagcctgtacgtgaagggcgagcccatcatcaacttctacgaccccctggtgttccctagcgacgagttcgacgctagcatcagccaagtgaacgagaagatcaatcagagcctggccttcatcagaaagagcgacgagctgctgcacaacgtgaacgccggcaagagcaccaccaacatcatgatcaccaccatcattatcgtgatcatcgtgattctcctgtccctgatcgccgtcggcctgctcctgtactgcaaggctagaagcacccccgtgaccctgagcaaggatcagctgagcggcatcaacaacatcgccttcagcaactga

SEQ ID NO: 15 - protein, 544 aa, synthetic construct
MELLILKANAITTILTAVTFCFASGQNCTEEFYQSTCSAVSKGYLSALRTGWYTCVITIELSNIKENKCNGTDAKVKLIKQELDKYKNAVTELQLLMQSTPPTNNRARRELPRFMNYTLNNAKKTNVTLSKKRKRRFLGFLLGVGSAIASGVAVSKVLHLEGEVNKIKSALLSTNKAVVSLSNGVSVCTSKVLDLKNYIDKQLLPIVNKQSCSISNIETVIEFQQKNNRLLEITREFSVNAGVTTPVSTYMLTNSELLSLINDMPITNDQKKLMSNNVQIVRQQSYSIMSIIKEEVLAYVVQLPLYGVIDTPCWKLHTSPLCTTNTKEGSNICLTRTDRGWYCDNAGSVSFFPQAETCKVQSNRVFCDTMNSLTLPSEINLCNVDIFNPKYDCKIMTSKTDVSSSVITSLGAIVSCYGKTKCTASNKNRGIIKTFSNGCDYVSNKGMDTVSVGNTLYYVNKQECKSLYVKGEPIINFYDPLVFPSDEFDASISQVNEKINQSLAFIRKSDELLSAIGGYIPEAPRDGQAYVRKDGEWVLLSTFL

SEQ ID NO: 16 - DNA, 1635 bp, synthetic construct
  source 1..1635: mol_type = other DNA
atggagctgctgatcctgaaggccaacgccatcaccaccatcctgaccgccgtgaccttctgcttcgctagcgggcagaactgcaccgaggagttctatcagagcacctgcagcgccgtcagcaaaggctacctgagcgccctgagaaccggctggtacacctgcgtgattaccatcgagctgagcaacatcaaggagaacaagtgcaacggcaccgacgccaaggtgaagctgatcaagcaagagctggacaagtacaagaacgccgtgaccgagctgcagctgctgatgcagagcaccccccccaccaacaacagagctagaagagagctgcctagattcatgaactacaccctgaacaacgccaagaagaccaacgtgaccctgagcaagaagagaaagagaagattcctgggcttcctgctgggcgtgggcagcgccattgctagcggcgtggccgtgagcaaggtgctgcacctcgagggcgaggtgaacaagatcaagagcgccctgctgtccaccaacaaggccgtggtgagcctgagcaacggcgtgagcgtgtgcacaagcaaggtcctggacctgaagaactacatcgacaagcagctgctgcccatcgtcaacaagcaatcctgcagcatcagcaacatcgagaccgtgatcgagtttcagcagaagaacaacagactgctggagatcacaagagagttcagcgtgaacgccggcgtgaccacccccgtgagcacctacatgctgaccaacagcgaactcctgagcctgatcaacgacatgcccatcaccaacgatcagaagaagctgatgagcaacaacgtgcagatcgtgagacagcagagctacagcatcatgagcatcatcaaggaagaggtgctggcctacgtggtgcagctgcccctgtacggcgtgatcgacaccccctgctggaagctgcacacaagccccctgtgcaccaccaacaccaaggagggcagcaacatctgcctgacaagaaccgacagaggctggtactgcgacaacgccggcagcgtgagcttcttcccccaagccgagacctgcaaggtgcagagcaacagagtgttctgcgacaccatgaacagcctgaccctgcctagcgagatcaacctgtgcaacgtggacatcttcaaccccaagtacgactgcaagatcatgacaagcaagaccgacgtgagcagcagcgtgatcacaagcctgggcgccatcgtgagctgctacggcaagaccaagtgcaccgctagcaacaagaacagaggcatcatcaagaccttcagcaacggctgcgactacgtgagcaacaagggcatggacaccgtgagcgtgggcaacaccctgtactacgtgaataaacaagagtgcaagagcctgtacgtgaagggcgagcccatcatcaacttctacgaccccctggtgttccctagcgacgagttcgacgctagcatcagccaagtgaacgagaagatcaatcagagcctggccttcatcagaaagagcgacgagctgctgagcgccatcggcggctacatccccgaggcccctagagacggccaagcctacgtgagaaaggacggcgagtgggtgctgctgagcaccttcctgtga

SEQ ID NO: 17 - protein, 574 aa, synthetic construct
MELLILKANAITTILTAVTFCFASGQNCTEEFYQSTCSAVSKGYLSALRTGWYTCVITIELSNIKENKCNGTDAKVKLIKQELDKYKNAVTELQLLMQSTPPTNNRARRELPRFMNYTLNNAKKTNVTLSKKRKRRFLGFLLGVGSAIASGVAVSKVLHLEGEVNKIKSALLSTNKAVVSLSNGVSVCTSKVLDLKNYIDKQLLPIVNKQSCSISNIETVIEFQQKNNRLLEITREFSVNAGVTTPVSTYMLTNSELLSLINDMPITNDQKKLMSNNVQIVRQQSYSIMSIIKEEVLAYVVQLPLYGVIDTPCWKLHTSPLCTTNTKEGSNICLTRTDRGWYCDNAGSVSFFPQAETCKVQSNRVFCDTMNSLTLPSEINLCNVDIFNPKYDCKIMTSKTDVSSSVITSLGAIVSCYGKTKCTASNKNRGIIKTFSNGCDYVSNKGMDTVSVGNTLYYVNKQECKSLYVKGEPIINFYDPLVFPSDEFDASISQVNEKINQSLAFIRKSDELLHNVNAGKSTTNIMITTIIIVIIVILLSLIAVGLLLYCKARSTPVTLSKDQLSGINNIAFSN

SEQ ID NO: 18 - DNA, 1725 bp, synthetic construct
  source 1..1725: mol_type = other DNA
atggagctgctgatcctgaaggccaacgccatcaccaccatcctgaccgccgtgaccttctgcttcgctagcgggcagaactgcaccgaggagttctatcagagcacctgcagcgccgtgagcaagggctacctgagcgccctgagaaccggctggtacacctgtgtcatcaccatcgagctgagcaacatcaaggagaacaagtgcaacggcaccgacgccaaggtgaagctgatcaagcaagagctggacaagtacaagaacgccgtgaccgagctgcagctgctgatgcagagcaccccccccaccaacaacagagctagaagagagctgcctagattcatgaactacaccctgaacaacgccaagaagaccaacgtgaccctgagcaagaaaagaaagagaagattcctggggttcctgctgggggtgggcagcgccattgctagcggcgtggccgtctccaaggtcctgcacctggagggcgaggtgaacaagatcaagagcgccctgctgagcaccaacaaggccgtggtgagcctgagcaacggcgtgagcgtgtgcacaagcaaggtgctggacctgaagaactacatcgacaagcagctgctgcccatcgtcaacaaacagtcctgcagcatcagcaacatcgagaccgtgatcgagtttcagcagaagaacaacagactgctggagatcacaagagagttcagcgtcaatgccggggtgaccacccccgtgagcacctacatgctgaccaacagcgagctgctgagcctcatcaacgacatgcccatcaccaacgatcagaagaagctgatgagcaacaacgtgcagatcgtgagacagcagagctacagcatcatgagcatcatcaaggaagaggtgctggcctacgtggtgcagctgcccctgtacggcgtgatcgacaccccctgctggaagctgcacacaagccccctgtgtaccaccaacaccaaagagggcagcaacatctgcctgacaagaaccgacagaggctggtactgcgacaacgccggcagcgtgagcttcttcccccaagccgagacctgcaaggtgcagagcaacagagtgttctgcgacaccatgaacagcctgaccctgcctagcgagatcaacctgtgcaacgtggacatcttcaaccccaagtacgactgcaagatcatgacaagcaagaccgacgtgagcagctccgtgatcacaagcctgggcgccatcgtgagctgctacggcaagaccaagtgcaccgctagcaacaagaacagaggcatcatcaagaccttcagcaacggctgcgactacgtgagcaacaagggcatggacaccgtgagcgtgggcaacaccctgtactacgtgaacaagcaagagtgcaagagcctgtacgtgaagggcgagcccatcatcaacttctacgaccccctggtgttccctagcgacgagttcgacgctagcatcagccaagtgaacgagaagatcaatcagagcctggccttcatcagaaagagcgacgagctgctgcacaacgtgaacgccggcaagagcaccaccaacatcatgatcacaaccatcattatcgtgatcatcgtgattctcctgagcctgatcgccgtgggcctgctcctgtactgcaaggctagaagcacccccgtgaccctgagcaaggatcagctgagcggcatcaacaacatcgccttcagcaactga

SEQ ID NO: 19 - protein, 502 aa, synthetic construct
MELLILKANAITTILTAVTFCFASGQNCTEEFYQSTCSAVSKGYLSALRTGWYTSVITIELSNIKENKCNGTDAKVKLIKQELDKYKNAVTELQLLMQSTPPTSAIASGVAVSKVLHLEGEVNKIKSALLSTNKAVVSLSNGVSVLTSKVLDLKNYIDKQLLPIVNKQSCSISNIETVIEFQQKNNRLLEITREFSVNAGVTTPVSTYMLTNSELLSLINDMPITNDQKKLMSNNVQIVRQQSYSIMSIIKEEVLAYVVQLPLYGVIDTPCWKLHTSPLCTTNTKEGSNICLTRTDRGWYCDNAGSVSFFPQAETCKVQSNRVFCDTMNSLTLPSEINLCNVDIFNPKYDCKIMTSKTDVSSSVITSLGAIVSCYGKTKCTASNKNRGIIKTFSNGCDYVSNKGMDTVSVGNTLYYVNKQECKSLYVKGEPIINFYDPLVFPSDEFDASISQVNEKINQSLAFIRKSDELLSAIGGYIPEAPRDGQAYVRKDGEWVLLSTFL

SEQ ID NO: 20 - DNA, 1509 bp, synthetic construct
  source 1..1509: mol_type = other DNA
atggagctgctgatcctgaaggccaacgccatcaccaccatcctgaccgccgtgaccttctgcttcgctagcgggcagaactgcaccgaggagttctatcagagcacctgcagcgctgtgagcaaaggctatctgagcgccctgagaaccggctggtacacaagcgtcatcaccatcgagctgagcaacatcaaggagaacaagtgcaacggcaccgacgccaaggtgaagctgatcaagcaagagctggacaagtacaagaacgccgtgaccgagctgcagctcctgatgcagagcaccccccctacctccgctattgctagcggcgtggccgtgagcaaggtcctgcacctggagggcgaggtgaacaagatcaagagcgccctgctcagcaccaacaaggccgtggtgagcctgagcaacggcgtgagcgtgctgacaagcaaggtgctggacctgaagaactacatcgacaagcagctgctgcccatcgtgaacaagcagagctgcagcatcagcaacatcgagaccgtgatcgagtttcagcagaagaacaacagactgctggagatcacaagagagttcagcgtgaacgccggcgtgaccacccccgtgagcacctacatgctgaccaacagcgaactgctgtccctgattaacgacatgcccatcaccaacgatcagaagaagctgatgagcaacaacgtgcagatcgtgagacagcagagctacagcatcatgagcatcatcaaggaagaggtgctggcctacgtggtgcagctgcccctgtacggcgtgatcgacaccccctgctggaagctgcacacaagccccctgtgcaccaccaacaccaaggagggcagcaacatctgcctgacaagaaccgacagaggctggtactgcgacaacgccggcagcgtgagcttcttcccccaagccgagacctgcaaggtgcagagcaacagagtgttctgcgacaccatgaacagcctgaccctgcctagcgagatcaacctgtgcaacgtggacatcttcaaccccaagtacgactgcaagatcatgacaagcaagaccgacgtgagcagcagcgtgatcacaagcctgggcgccatcgtgagctgctacggcaagaccaagtgcaccgctagcaacaagaacagaggcatcatcaagaccttcagcaacggctgcgactacgtgagcaacaagggcatggacaccgtgagcgtgggcaacaccctgtactacgtcaacaagcaagagtgtaagagcctgtacgtgaagggcgagcccatcatcaacttctacgaccccctggtgttccctagcgacgagttcgacgctagcatcagccaagtgaacgagaagatcaatcagagcctggccttcatcagaaagagcgacgagctgctgagcgctatcggcggctacatccccgaggcccctagagacggccaagcctacgtgagaaaggacggcgagtgggtgctgctgtccaccttcctctga

SEQ ID NO: 21 - protein, 532 aa, synthetic construct
MELLILKANAITTILTAVTFCFASGQNCTEEFYQSTCSAVSKGYLSALRTGWYTSVITIELSNIKENKCNGTDAKVKLIKQELDKYKNAVTELQLLMQSTPPTSAIASGVAVSKVLHLEGEVNKIKSALLSTNKAVVSLSNGVSVLTSKVLDLKNYIDKQLLPIVNKQSCSISNIETVIEFQQKNNRLLEITREFSVNAGVTTPVSTYMLTNSELLSLINDMPITNDQKKLMSNNVQIVRQQSYSIMSIIKEEVLAYVVQLPLYGVIDTPCWKLHTSPLCTTNTKEGSNICLTRTDRGWYCDNAGSVSFFPQAETCKVQSNRVFCDTMNSLTLPSEINLCNVDIFNPKYDCKIMTSKTDVSSSVITSLGAIVSCYGKTKCTASNKNRGIIKTFSNGCDYVSNKGMDTVSVGNTLYYVNKQECKSLYVKGEPIINFYDPLVFPSDEFDASISQVNEKINQSLAFIRKSDELLHNVNAGKSTTNIMITTIIIVIIVILLSLIAVGLLLYCKARSTPVTLSKDQLSGINNIAFSN

SEQ ID NO: 22 - DNA, 1599 bp, synthetic construct
  source 1..1599: mol_type = other DNA
atggagctgctgatcctgaaggccaacgccatcacaaccatcctgaccgccgtgaccttctgcttcgctagcgggcagaactgcaccgaggagttctatcagagcacctgcagcgccgtgagcaaggggtatctgagcgccctgagaaccggctggtacacctccgtcatcaccatcgagctgagcaacatcaaggagaacaagtgcaacggcaccgacgccaaggtgaagctgatcaagcaagagctggacaagtacaagaacgccgtgaccgagctgcaactgctgatgcaaagcacccctcccacaagcgccatcgcctccggcgtggctgtcagcaaggtcctccatctggagggcgaggtgaacaagatcaagagcgccctgctgagcaccaacaaggccgtggtgagcctgagcaacggcgtgagcgtgctgacctccaaggtgctggatctgaagaactacatcgacaagcagctgctgcccatcgtgaacaagcagagctgcagcatcagcaacatcgagaccgtgatcgagtttcagcagaagaacaacagactgctggagatcacaagagagttcagcgtgaatgctggcgtcaccacccccgtgagcacctacatgctgaccaacagcgagctgctgagcctgatcaacgacatgcccatcaccaacgatcagaagaagctgatgagcaacaacgtgcagatcgtgagacagcagagctacagcatcatgagcatcatcaaggaagaggtgctggcctacgtggtgcagctgcccctgtacggcgtgatcgacaccccctgctggaagctgcacacaagccccctgtgcacaaccaacaccaaggagggcagcaacatctgcctgacaagaaccgacagaggctggtactgcgacaacgccggcagcgtgagcttcttcccccaagccgagacctgcaaggtgcagagcaacagagtgttctgcgacaccatgaacagcctgaccctgcctagcgagatcaacctgtgcaacgtggacatcttcaaccccaagtacgactgcaagatcatgacaagcaagaccgacgtgagcagcagcgtgattacaagcctgggcgccatcgtgagctgctacggcaagaccaagtgcaccgctagcaacaagaacagaggcatcatcaagaccttcagcaacggctgcgactacgtgagcaacaagggcatggacaccgtgagcgtgggcaacaccctgtactacgtgaataagcaagagtgcaagagcctgtacgtgaagggcgagcccatcatcaacttctacgaccccctggtgttccctagcgacgagttcgacgctagcatcagccaagtgaacgagaagatcaatcagagcctggccttcatcagaaagagcgacgagctgctgcacaacgtgaacgccggcaagagcaccaccaacatcatgatcaccaccatcattatcgtgatcatcgtgattctcctgtccctgatcgccgtcggcctgctcctgtactgcaaggctagaagcacccccgtgaccctgagcaaggatcagctgagcggcatcaacaacatcgccttcagcaactga

SEQ ID NO: 23 - protein, 502 aa, synthetic construct
MELLIHRSSAIFLTLAVNALYLTSSQNITEEFYQSTCSAVSRGYFSALRTGWYTSVITIELSNIKETKCNGTDTKVKLIKQELDKYKNAVTELQLLMQNTPAASAIASGIAVSKVLHLEGEVNKIKNALLSTNKAVVSLSNGVSVLTSKVLDLKNYINNRLLPIVNQQSCRISNIETVIEFQQMNSRLLEITREFSVNAGVTTPLSTYMLTNSELLSLINDMPITNDQKKLMSSNVQIVRQQSYSIMSIIKEEVLAYVVQLPIYGVIDTPCWKLHTSPLCTTNIKEGSNICLTRTDRGWYCDNAGSVSFFPQADTCKVQSNRVFCDTMNSLTLPSEVSLCNTDIFNSKYDCKIMTSKTDISSSVITSLGAIVSCYGKTKCTASNKNRGIIKTFSNGCDYVSNKGVDTVSVGNTLYYVNKLEGKNLYVKGEPIINYYDPLVFPSDEFDASISQVNEKINQSLAFIRRSDELLSAIGGYIPEAPRDGQAYVRKDGEWVLLSTFL

SEQ ID NO: 24 - DNA, 1509 bp, synthetic construct
  source 1..1509: mol_type = other DNA
atggagctgctgatccacagaagcagcgccatcttcctgaccctggccgtgaacgccctgtacctgacaagcagccaaaacatcaccgaggagttctatcagagcacctgcagcgccgtgagcagaggctacttcagcgccctgagaaccggctggtacacctccgtgatcacaatcgaactgagcaacattaaggagaccaagtgtaacggcaccgacaccaaggtgaagctgatcaagcaagagctggacaagtacaagaacgccgtgaccgagctgcagctgctgatgcagaacacccccgccgctagcgccatcgctagcggcatcgccgtgtccaaagtgctgcacctggagggcgaggtgaacaagatcaagaacgccctgctgagcacaaacaaggccgtggtgagcctgagcaacggcgtgagcgtgctgacaagcaaggtgctggacctgaagaactacatcaacaacagactgctgcccatcgtgaatcagcagagctgcagaatcagcaacatcgagaccgtgatcgagtttcagcagatgaacagcagactgctggagatcacaagagagttcagcgtgaacgccggcgtgaccacccccctgagcacctacatgctgaccaacagcgaactgctgagcctgatcaacgacatgcccatcaccaacgatcagaagaagctgatgagcagcaacgtgcagatcgtgagacagcagagctacagcatcatgagcatcatcaaggaagaggtgctggcctacgtggtgcagctgcccatctacggcgtgatcgacaccccctgctggaagctgcacacaagccccctgtgcaccaccaatatcaaggagggcagcaacatctgcctgacaagaaccgacagaggctggtactgcgacaacgccggcagcgtgagcttcttcccccaagccgacacctgcaaggtgcagagcaacagagtgttctgcgacaccatgaacagcctgaccctgcctagcgaggtgagcctgtgcaacaccgacatcttcaacagcaagtacgactgcaagatcatgacaagcaagaccgacatcagcagcagcgtgatcacaagcctgggcgccatcgtgagctgctacggcaagacaaagtgcacagctagcaacaagaacagaggcatcatcaagaccttcagcaacggctgcgactacgtgagcaacaagggcgtggacaccgtgagcgtgggcaacaccctgtactacgtgaacaagctggagggcaagaacctgtacgtgaagggcgagcccatcatcaactactacgaccccctggtgttccctagcgacgagttcgacgctagcatcagccaagtgaacgagaagatcaatcagagcctggccttcatcagaagaagcgacgagctgctcagcgctatcggcggctacatccccgaggcccctagagacggccaagcctacgtgagaaaggacggcgagtgggtgctcctgagcaccttcctctga

SEQ ID NO: 25 - protein, 532 aa, synthetic construct
MELLIHRSSAIFLTLAVNALYLTSSQNITEEFYQSTCSAVSRGYFSALRTGWYTSVITIELSNIKETKCNGTDTKVKLIKQELDKYKNAVTELQLLMQNTPAASAIASGIAVSKVLHLEGEVNKIKNALLSTNKAVVSLSNGVSVLTSKVLDLKNYINNRLLPIVNQQSCRISNIETVIEFQQMNSRLLEITREFSVNAGVTTPLSTYMLTNSELLSLINDMPITNDQKKLMSSNVQIVRQQSYSIMSIIKEEVLAYVVQLPIYGVIDTPCWKLHTSPLCTTNIKEGSNICLTRTDRGWYCDNAGSVSFFPQADTCKVQSNRVFCDTMNSLTLPSEVSLCNTDIFNSKYDCKIMTSKTDISSSVITSLGAIVSCYGKTKCTASNKNRGIIKTFSNGCDYVSNKGVDTVSVGNTLYYVNKLEGKNLYVKGEPIINYYDPLVFPSDEFDASISQVNEKINQSLAFIRRSDELLHNVNTGKSTTNIMITTIIIVIIVVLLSLIAIGLLLYCKAKNTPVTLSKDQLSGINNIAFSK

SEQ ID NO: 26 - DNA, 1599 bp, synthetic construct
  source 1..1599: mol_type = other DNA
atggagctgctgatccacagaagcagcgccatcttcctgaccctggccgtgaacgccctgtacctgacaagcagccaaaacatcaccgaggagttctatcagagcacctgcagcgccgtgagcagaggctacttcagcgccctgagaaccggctggtacacaagcgtcatcaccatcgagctgagcaatattaaggagaccaagtgtaatggcaccgacaccaaggtgaagctgatcaagcaagagctggacaagtacaagaacgccgtgaccgagctgcagctgctgatgcagaacacccctgccgctagcgccatcgctagcggcatcgccgtgagcaaagtgctgcatctggagggcgaggtgaacaagatcaagaacgccctgctgagcaccaacaaggccgtggtgagcctgagcaacggcgtgagcgtgctgacctccaaggtgctggacctcaagaactacatcaacaacagactgctgcccatcgtgaatcagcagagctgcagaatcagcaacatcgagaccgtgatcgagtttcagcagatgaacagcagactgctggagatcacaagagagttcagcgtgaacgccggcgtgaccacccccctgagcacctacatgctgaccaacagcgagctgctgagcctgatcaacgacatgcccatcaccaacgatcagaagaagctgatgagcagcaacgtgcagatcgtgagacagcagagctacagcatcatgagcatcatcaaggaagaggtgctggcctacgtggtgcagctgcccatctacggcgtgatcgacaccccctgctggaagctgcacacaagccccctgtgcaccaccaacatcaaagagggctccaacatctgcctgacaagaaccgacagaggctggtactgcgacaacgccggcagcgtgagcttcttcccccaagccgacacctgcaaggtgcagagcaacagagtgttctgcgacaccatgaacagcctgaccctgcctagcgaggtgagcctgtgcaacaccgacatcttcaacagcaagtacgactgcaagatcatgacaagcaagaccgacatcagcagcagcgtgatcacaagcctgggcgccatcgtgagctgctacggcaagaccaagtgcaccgctagcaacaagaacagaggcatcatcaagaccttcagcaacggctgcgactacgtgagcaacaagggcgtggacaccgtgagcgtgggcaacaccctgtactacgtgaacaagctggagggcaagaacctgtacgtgaagggcgagcccatcatcaactactacgaccccctggtgttccctagcgacgagttcgacgctagcatcagccaagtgaacgagaagatcaatcagagcctggccttcatcagaagaagcgacgagctgctgcacaacgtgaacaccggcaagtccaccacaaacatcatgatcaccaccatcattatcgtgatcatcgtggtgctgctgtccctgatcgccatcggcctgctcctgtactgcaaggccaagaacacacctgtgaccctgagcaaggatcagctgagcggcatcaacaacatcgccttcagcaagtga

SEQ ID NO: 27 - protein, 544 aa, synthetic construct
MELLIHRSSAIFLTLAVNALYLTSSQNCTEEFYQSTCSAVSRGYFSALRTGWYTCVITIELSNIKETKCNGTDTKVKLIKQELDKYKNAVTELQLLMQNTPAANNRARREAPQYMNYTINTTKNLNVSISKKRKRRFLGFLLGVGSAIASGIAVSKVLHLEGEVNKIKNALLSTNKAVVSLSNGVSVCTSKVLDLKNYINNRLLPIVNQQSCRISNIETVIEFQQMNSRLLEITREFSVNAGVTTPLSTYMLTNSELLSLINDMPITNDQKKLMSSNVQIVRQQSYSIMSIIKEEVLAYVVQLPIYGVIDTPCWKLHTSPLCTTNIKEGSNICLTRTDRGWYCDNAGSVSFFPQADTCKVQSNRVFCDTMNSLTLPSEVSLCNTDIFNSKYDCKIMTSKTDISSSVITSLGAIVSCYGKTKCTASNKNRGIIKTFSNGCDYVSNKGVDTVSVGNTLYYVNKLECKNLYVKGEPIINYYDPLVFPSDEFDASISQVNEKINQSLAFIRRSDELLSAIGGYIPEAPRDGQAYVRKDGEWVLLSTFL

SEQ ID NO: 28 - DNA, 1635 bp, synthetic construct
  source 1..1635: mol_type = other DNA
atggagctgctgatccacagaagcagcgccatcttcctgaccctggccgtgaacgccctgtacctgacaagcagccaaaactgcaccgaggagttctatcagagcacctgcagcgccgtgagcagaggctacttcagcgccctgagaaccggctggtacacctgcgtcatcacaatcgagctgagcaacatcaaagagaccaagtgcaacggcaccgacaccaaggtgaagctgatcaagcaagagctggacaagtacaagaacgccgtgaccgagctgcagctgctgatgcagaacacccccgccgccaacaacagagctagaagagaggcccctcagtacatgaactacaccatcaacaccaccaagaacctgaacgtgagcatcagcaagaagagaaagagaagattcctgggcttcctgctgggcgtgggcagcgccatcgctagcggcatcgccgtgtccaaggtcctgcatctcgagggcgaggtgaacaagatcaagaacgccctgctgagcacaaacaaggccgtggtgagcctgagcaacggcgtgagcgtgtgcacaagcaaggtgctggacctcaagaactacatcaacaacagactgctgcccatcgtgaatcagcagagctgcagaatcagcaacatcgagaccgtgatcgagtttcagcagatgaacagcagactgctggagatcacaagagagttcagcgtgaacgccggcgtgaccacccccctgagcacctacatgctgaccaacagcgagctgctgagcctcatcaacgacatgcccatcaccaacgatcagaagaagctgatgagcagcaacgtgcagatcgtgagacagcagagctacagcatcatgagcatcatcaaggaagaggtgctggcctacgtggtgcagctgcccatctacggcgtgatcgacaccccctgctggaagctgcacacaagccccctgtgcaccaccaacatcaaggagggcagcaacatctgcctgacaagaaccgacagaggctggtactgcgacaacgccggcagcgtgagcttcttcccccaagccgacacctgcaaggtgcagagcaacagagtgttctgcgacaccatgaacagcctgaccctgcctagcgaggtgagcctgtgcaacaccgacatcttcaacagcaagtacgactgcaagatcatgacaagcaagaccgacatcagcagcagcgtcatcacaagcctgggcgccatcgtgagctgctacggcaagaccaaatgtaccgctagcaacaagaacagaggcatcatcaagaccttcagcaacggctgcgactacgtgagcaacaagggcgtggacaccgtgagcgtgggcaacaccctgtactacgtgaacaagctggagtgcaagaacctgtacgtgaagggcgagcccatcatcaactactacgaccccctggtgttccctagcgacgagttcgacgctagcatcagccaagtgaacgagaagatcaatcagagcctggccttcatcagaagaagcgacgaactgctgagcgccattggcggctacatccccgaggcccctagagacggccaagcctacgtgagaaaggacggcgagtgggtgctgctgagcaccttcctgtga

SEQ ID NO: 29 - protein, 574 aa, synthetic construct
MELLIHRSSAIFLTLAVNALYLTSSQNCTEEFYQSTCSAVSRGYFSALRTGWYTCVITIELSNIKETKCNGTDTKVKLIKQELDKYKNAVTELQLLMQNTPAANNRARREAPQYMNYTINTTKNLNVSISKKRKRRFLGFLLGVGSAIASGIAVSKVLHLEGEVNKIKNALLSTNKAVVSLSNGVSVCTSKVLDLKNYINNRLLPIVNQQSCRISNIETVIEFQQMNSRLLEITREFSVNAGVTTPLSTYMLTNSELLSLINDMPITNDQKKLMSSNVQIVRQQSYSIMSIIKEEVLAYVVQLPIYGVIDTPCWKLHTSPLCTTNIKEGSNICLTRTDRGWYCDNAGSVSFFPQADTCKVQSNRVFCDTMNSLTLPSEVSLCNTDIFNSKYDCKIMTSKTDISSSVITSLGAIVSCYGKTKCTASNKNRGIIKTFSNGCDYVSNKGVDTVSVGNTLYYVNKLECKNLYVKGEPIINYYDPLVFPSDEFDASISQVNEKINQSLAFIRRSDELLHNVNTGKSTTNIMITTIIIVIIVVLLSLIAIGLLLYCKAKNTPVTLSKDQLSGINNIAFSK

SEQ ID NO: 30 - DNA, 1725 bp, synthetic construct
  source 1..1725: mol_type = other DNA
atggagctgctgatccacagaagcagcgccatcttcctgaccctggccgtgaacgccctgtacctgacaagcagccaaaactgcaccgaggagttctatcagagcacctgcagcgccgtgagcagaggctacttcagcgccctgagaaccggctggtacacctgtgtgatcaccatcgagctgagcaacatcaaggagaccaaatgtaacggcaccgacaccaaggtgaagctgatcaagcaagagctggacaagtacaagaacgccgtgaccgagctgcagctgctgatgcagaacacccctgccgccaacaacagagctagaagagaggcccctcagtacatgaactacaccatcaacaccaccaagaacctgaacgtgagcatcagcaagaagagaaagagaagattcctgggcttcctgctgggcgtgggcagcgccatcgctagcggcatcgccgtgagcaaggtgctgcacctggagggcgaggtgaacaagatcaagaacgccctgctgagcaccaacaaggccgtggtgagcctgagcaacggcgtgagcgtgtgcacaagcaaagtgctggacctcaagaactacatcaacaacagactgctgcccatcgtgaatcagcagagctgcagaatcagcaacatcgagaccgtgatcgagtttcagcagatgaacagcagactgctggagatcacaagagagttcagcgtgaacgccggcgtgaccacccccctgagcacctacatgctgaccaacagcgaactgctcagcctgattaatgacatgcccatcaccaacgatcagaagaagctgatgagcagcaacgtgcagatcgtgagacagcagagctacagcatcatgagcatcatcaaggaagaggtgctggcctacgtggtgcagctgcccatctacggcgtgatcgacaccccctgctggaagctgcacacaagccccctgtgcaccaccaacattaaagaggggagcaacatctgcctgacaagaaccgacagaggctggtactgcgacaacgccggcagcgtgagcttcttcccccaagccgacacctgcaaggtgcagagcaacagagtgttctgcgacaccatgaacagcctgaccctgcctagcgaggtgagcctgtgcaacaccgacatcttcaacagcaagtacgactgcaagatcatgacaagcaagaccgacatcagcagcagcgtgatcacaagcctcggcgccatcgtgagctgctacggcaagaccaagtgcaccgctagcaacaagaacagaggcatcatcaagaccttcagcaacggctgcgactacgtgagcaacaagggcgtggacaccgtgagcgtgggcaacaccctgtactacgtgaacaagctggagtgcaagaacctgtacgtgaagggcgagcccatcatcaactactacgaccccctggtgttccctagcgacgagttcgacgctagcatcagccaagtgaacgagaagatcaatcagagcctggccttcatcagaagaagcgacgagctgctgcacaacgtgaacaccggcaagagcaccacaaatatcatgatcaccaccatcattatcgtgatcatcgtggtgctcctgagcctgatcgccatcggcctgctcctgtactgcaaggccaaaaacacccccgtgacactgagcaaggatcagctgagcggcatcaacaacatcgccttcagcaagtga

SEQ ID NO: 31 - protein, 502 aa, synthetic construct
MELLIHRSSAIFLTLAVNALYLTSSQNCTEEFYQSTCSAVSRGYFSALRTGWYTSVITIELSNIKETKCNGTDTKVKLIKQELDKYKNAVTELQLLMQNTPAASAIASGIAVSKVLHLEGEVNKIKNALLSTNKAVVSLSNGVSVLTSKVLDLKNYINNRLLPIVNQQSCRISNIETVIEFQQMNSRLLEITREFSVNAGVTTPLSTYMLTNSELLSLINDMPITNDQKKLMSSNVQIVRQQSYSIMSIIKEEVLAYVVQLPIYGVIDTPCWKLHTSPLCTTNIKEGSNICLTRTDRGWYCDNAGSVSFFPQADTCKVQSNRVFCDTMNSLTLPSEVSLCNTDIFNSKYDCKIMTSKTDISSSVITSLGAIVSCYGKTKCTASNKNRGIIKTFSNGCDYVSNKGVDTVSVGNTLYYVNKLECKNLYVKGEPIINYYDPLVFPSDEFDASISQVNEKINQSLAFIRRSDELLSAIGGYIPEAPRDGQAYVRKDGEWVLLSTFL

SEQ ID NO: 32 - DNA, 1509 bp, synthetic construct
  source 1..1509: mol_type = other DNA
atggagctgctgatccacagaagcagcgccatcttcctgaccctggccgtgaacgccctgtacctgacaagcagccaaaactgcaccgaggagttctatcagagcacctgcagcgccgtgagcagaggctacttcagcgccctgagaaccggctggtacacctccgtgatcacaatcgaactgagcaacattaaggagaccaagtgtaacggcaccgacaccaaggtgaagctgatcaagcaagagctggacaagtacaagaacgccgtgaccgagctgcagctgctgatgcagaacacccccgccgctagcgccatcgctagcggcatcgccgtgtccaaagtgctgcacctggagggcgaggtgaacaagatcaagaacgccctgctgagcacaaacaaggccgtggtgagcctgagcaacggcgtgagcgtgctgacaagcaaggtgctggacctgaagaactacatcaacaacagactgctgcccatcgtgaatcagcagagctgcagaatcagcaacatcgagaccgtgatcgagtttcagcagatgaacagcagactgctggagatcacaagagagttcagcgtgaacgccggcgtgaccacccccctgagcacctacatgctgaccaacagcgaactgctgagcctgatcaacgacatgcccatcaccaacgatcagaagaagctgatgagcagcaacgtgcagatcgtgagacagcagagctacagcatcatgagcatcatcaaggaagaggtgctggcctacgtggtgcagctgcccatctacggcgtgatcgacaccccctgctggaagctgcacacaagccccctgtgcaccaccaatatcaaggagggcagcaacatctgcctgacaagaaccgacagaggctggtactgcgacaacgccggcagcgtgagcttcttcccccaagccgacacctgcaaggtgcagagcaacagagtgttctgcgacaccatgaacagcctgaccctgcctagcgaggtgagcctgtgcaacaccgacatcttcaacagcaagtacgactgcaagatcatgacaagcaagaccgacatcagcagcagcgtgatcacaagcctgggcgccatcgtgagctgctacggcaagacaaagtgcacagctagcaacaagaacagaggcatcatcaagaccttcagcaacggctgcgactacgtgagcaacaagggcgtggacaccgtgagcgtgggcaacaccctgtactacgtgaacaagctggagtgcaagaacctgtacgtgaagggcgagcccatcatcaactactacgaccccctggtgttccctagcgacgagttcgacgctagcatcagccaagtgaacgagaagatcaatcagagcctggccttcatcagaagaagcgacgagctgctcagcgctatcggcggctacatccccgaggcccctagagacggccaagcctacgtgagaaaggacggcgagtgggtgctcctgagcaccttcctctga

SEQ ID NO: 33 - protein, 532 aa, synthetic construct
MELLIHRSSAIFLTLAVNALYLTSSQNCTEEFYQSTCSAVSRGYFSALRTGWYTSVITIELSNIKETKCNGTDTKVKLIKQELDKYKNAVTELQLLMQNTPAASAIASGIAVSKVLHLEGEVNKIKNALLSTNKAVVSLSNGVSVLTSKVLDLKNYINNRLLPIVNQQSCRISNIETVIEFQQMNSRLLEITREFSVNAGVTTPLSTYMLTNSELLSLINDMPITNDQKKLMSSNVQIVRQQSYSIMSIIKEEVLAYVVQLPIYGVIDTPCWKLHTSPLCTTNIKEGSNICLTRTDRGWYCDNAGSVSFFPQADTCKVQSNRVFCDTMNSLTLPSEVSLCNTDIFNSKYDCKIMTSKTDISSSVITSLGAIVSCYGKTKCTASNKNRGIIKTFSNGCDYVSNKGVDTVSVGNTLYYVNKLECKNLYVKGEPIINYYDPLVFPSDEFDASISQVNEKINQSLAFIRRSDELLHNVNTGKSTTNIMITTIIIVIIVVLLSLIAIGLLLYCKAKNTPVTLSKDQLSGINNIAFSK

SEQ ID NO: 34 - DNA, 1599 bp, synthetic construct
  source 1..1599: mol_type = other DNA
atggagctgctgatccacagaagcagcgccatcttcctgaccctggccgtgaacgccctgtacctgacaagcagccaaaactgcaccgaggagttctatcagagcacctgcagcgccgtgagcagaggctacttcagcgccctgagaaccggctggtacacaagcgtcatcaccatcgagctgagcaatattaaggagaccaagtgtaatggcaccgacaccaaggtgaagctgatcaagcaagagctggacaagtacaagaacgccgtgaccgagctgcagctgctgatgcagaacacccctgccgctagcgccatcgctagcggcatcgccgtgagcaaagtgctgcatctggagggcgaggtgaacaagatcaagaacgccctgctgagcaccaacaaggccgtggtgagcctgagcaacggcgtgagcgtgctgacctccaaggtgctggacctcaagaactacatcaacaacagactgctgcccatcgtgaatcagcagagctgcagaatcagcaacatcgagaccgtgatcgagtttcagcagatgaacagcagactgctggagatcacaagagagttcagcgtgaacgccggcgtgaccacccccctgagcacctacatgctgaccaacagcgagctgctgagcctgatcaacgacatgcccatcaccaacgatcagaagaagctgatgagcagcaacgtgcagatcgtgagacagcagagctacagcatcatgagcatcatcaaggaagaggtgctggcctacgtggtgcagctgcccatctacggcgtgatcgacaccccctgctggaagctgcacacaagccccctgtgcaccaccaacatcaaagagggctccaacatctgcctgacaagaaccgacagaggctggtactgcgacaacgccggcagcgtgagcttcttcccccaagccgacacctgcaaggtgcagagcaacagagtgttctgcgacaccatgaacagcctgaccctgcctagcgaggtgagcctgtgcaacaccgacatcttcaacagcaagtacgactgcaagatcatgacaagcaagaccgacatcagcagcagcgtgatcacaagcctgggcgccatcgtgagctgctacggcaagaccaagtgcaccgctagcaacaagaacagaggcatcatcaagaccttcagcaacggctgcgactacgtgagcaacaagggcgtggacaccgtgagcgtgggcaacaccctgtactacgtgaacaagctggagtgcaagaacctgtacgtgaagggcgagcccatcatcaactactacgaccccctggtgttccctagcgacgagttcgacgctagcatcagccaagtgaacgagaagatcaatcagagcctggccttcatcagaagaagcgacgagctgctgcacaacgtgaacaccggcaagtccaccacaaacatcatgatcaccaccatcattatcgtgatcatcgtggtgctgctgtccctgatcgccatcggcctgctcctgtactgcaaggccaagaacacacctgtgaccctgagcaaggatcagctgagcggcatcaacaacatcgccttcagcaagtga

SEQ ID NO: 35 - DNA, 22 bp, synthetic construct
  source 1..22: mol_type = other DNA
acgtgggtataagaggcgcgac

SEQ ID NO: 36 - DNA, 27 bp, synthetic construct
  source 1..27: mol_type = other DNA
cttcggatcttcgatgctagacgatcc

SEQ ID NO: 37 - DNA, 27 bp, synthetic construct
  source 1..27: mol_type = other DNA
ctcctaattatgatgtgcagaaacaca

SEQ ID NO: 38 - DNA, 27 bp, synthetic construct
  source 1..27: mol_type = other DNA
ccagtgaatttatgattagcatcttct

SEQ ID NO: 39 - DNA, 20 bp, synthetic construct
  source 1..20: mol_type = other DNA
ataacatgccacataactta